European Patent Application EP 4 389 876 A1, published June 26, 2024. Title: METHOD FOR PREPARING RENAL PODOCYTES BY DISCONTINUOUS DIFFERENTIATION. Applicant: Guangzhou Asia Kidney Rebuilding Medical Technology Ltd. Application EP. The sequence listing filed with the application follows.

SEQUENCE LISTING (14 sequences)

SEQ ID NO: 1 - DNA, 20 bp, synthetic construct
  source 1..20: mol_type = other DNA
tgtttgggattgggaggctt

SEQ ID NO: 2 - DNA, 22 bp, synthetic construct
  source 1..22: mol_type = other DNA
gcacaaccaacaaattagggga

SEQ ID NO: 3 - DNA, 20 bp, synthetic construct
  source 1..20: mol_type = other DNA
tgagtttgagaggcgacacg

SEQ ID NO: 4 - DNA, 20 bp, synthetic construct
  source 1..20: mol_type = other DNA
tgcagtgcatatccatgggg

SEQ ID NO: 5 - DNA, 20 bp, synthetic construct
  source 1..20: mol_type = other DNA
cacggtgtcttcagaggcat

SEQ ID NO: 6 - DNA, 20 bp, synthetic construct
  source 1..20: mol_type = other DNA
acacatgaaggggcgtttct

SEQ ID NO: 7 - DNA, 20 bp, synthetic construct
  source 1..20: mol_type = other DNA
tctaccatggctacctgcct

SEQ ID NO: 8 - DNA, 20 bp, synthetic construct
  source 1..20: mol_type = other DNA
ggcaggctccttgataggtg

SEQ ID NO: 9 - DNA, 22 bp, synthetic construct
  source 1..22: mol_type = other DNA
cttgaatcccgaatggaaaggg

SEQ ID NO: 10 - DNA, 23 bp, synthetic construct
  source 1..23: mol_type = other DNA
gtgtatatcccagggtgatcctc

SEQ ID NO: 11 - DNA, 21 bp, synthetic construct
  source 1..21: mol_type = other DNA
tcaccgtgaatgttctgttcc

SEQ ID NO: 12 - DNA, 21 bp, synthetic construct
  source 1..21: mol_type = other DNA
agtgtggctaagggattaccc

SEQ ID NO: 13 - DNA, 19 bp, synthetic construct
  source 1..19: mol_type = other DNA
gtggtggacgtggatgagg

SEQ ID NO: 14 - DNA, 21 bp, synthetic construct
  source 1..21: mol_type = other DNA
ccggaggatttggtaccttcc